European Patent Specification EP 3 802 784 B1, published August 7, 2024. Title: OVER-EXPRESSION OF TRANSCRIPTIONAL ACTIVATOR/REPRESSOR GIS1 IN YEAST FOR INCREASED ETHANOL PRODUCTION. Applicant: Danisco US Inc. The sequence listing filed with the application follows.

SEQUENCE LISTING (5 sequences)

SEQ ID NO: 1 - DNA, 9 bp, Artificial Sequence
  Artificial element
tatagggat

SEQ ID NO: 2 - DNA, 2685 bp, Saccharomyces cerevisiae
atggaaatcaagccagtcgaagttatcgacggtgttccagtcttcaagccatctatgatggaatttgccaattttcaatacttcattgacgaaatcaccaagtttggtatcgaaaacggtattgtcaaggttattcctcccaaggaatggctggaattgttggaaggttctccacctgctgaatccttgaagactatccaactagattctccaattcaacagcaagccaagagatgggacaaacacgaaaacggtgtcttttccatcgaaaacgaatacgacaacaagtcttacaacttgacacaatggaagaatttggctgaatccttggattctagaatcagtcaaggtgacttcaacgacaagaccttaaaggaaaactgcagagtcgattctcaacaggattgttacgatttggctcaattacaaatcttggaatccgacttctggaagaccattgccttttccaagccattctacgctgttgacgaaaactcttccatcttcccatacgacttgactttatggaacttgaacaatttgccagattctatcaactccagcaacagacgtttgctaactggtcaatccaagtgtatctttccatggcacttggacgaacaaaacaagtgttctatcaactacttgcacttcggtgctccaaagcaatggtactccattccatctgccaacaccgatcaattcttgaagatcctatccaaggaaccatcaagcaacaaggaaaattgtccagctttcatccgtcatcaaaacatcattacttctccagactttttgagaaagaacaatatcaagttcaacagagttgtccaatttcaacatgaatttatcattacctttccttactgtatgtactccggtttcaactacggttacaactttggcgaatctatcgagttcatcttagatcagcaagctgttgtcagaaagcaaccattgaagtgtggttgcggcaacaagaaagaagagagaaagtctggtccattttccaacttgtcttacgactccaacgaaagcgaacaacgtggttctattaccgacaacgacaatgatttgtttcaaaaggtcagatccttcgacgaattgctaaaccactcctctcaagaattgcaaaacttggaagacaacaagaatccattgttttccaacatcaatatgaacagaccacaaagctcctctttgaggtctactacaccaaacggtgtcaaccaattcttgaacatgaatcaaactaccatcagcagaatttcctctccattgttatcaagaatgatggacttgtccaacatcgtggaaccaaccttggacgatcctggttccaagttcaagagaaaggttttgactccacaattaccacaaatgaacattccatccaactcttccaactttggtactccttctttgaccaatacaaactccttgctatcaaacatcactgctacatctaccaatccatccaccactaccaacggctctcaaaaccacaacaatgtcaacgccaatggtatcaacacctctgctgccgcttccatcaacaataacatttcctctaccaacaattctgccaataacagctcttccaacaataacgtttctactgttccatcttccatgatgcactcttccaccttgaatggtacttctggtttgggtggcgacaacgatgacaacatgttagctttgagcctagctaccttggccaacagtgctactgcttctccaagattgaccttaccacctttgtcttcaccaatgaatcccaacggtcacacttcctacaacggtaacatgatgaacaataactctggtaacggttccaacggtagcaactcttactccaatggtgtcaccactgctgccgctaccactacatctgctccacacaacttgtccatcgtttctccaaaccctacctacagtccaaatcccttgtctctatacttgaccaactccaagaatccattgaactctggtttggctccattatctccttccacttctaacattccattcttgaagagaaacaatgtcgttaccctaaacatctccagagaagcctccaagtctccaatctcttcctttgtcaacgactaccgttctccattgggtgtttccaatccattgatgtactcttccactatcaacgattactccaacggtactggtatccgtcaaaacagcaacaacatcaatccattggacgctggtccatctttttctcctttgcacaagaaaccaaagattttgaacggcaatgacaactccaatttggacagcaacaatttcgattactcttttactggtaacaagcaagaatccaatccatctatcttgaacaacaataccaacaataacgacaactacagaacttcttccatgaacaacaatggtaacaattaccaagctcactcttccaagtttggtgaaaacgaagtcatcatgtccgatcacggtaagatttacatctgtagagaatgtaacagacaattttcctctggtcaccatctaaccagacacaaaaagtcagttcattctggtgaaaagccacactcttgtccaagatgtggtaaaagattcaagagaagagatcatgtcttgcaacacttgaacaagaaaatcccatgcactcaagaaatggaaaacaccaagttggctgaatcttaa

SEQ ID NO: 3 - DNA, 757 bp, Artificial Sequence
  Artificial promoter
aatagagtatgattattttttttatattttttttttttggaaaacaaaattcttatagtaaagtaaggaatagtagcagaatatttttctgaagtgtttataataaagggagaaccgggaaagtagcaaaatgattggttaatttatgcaaatcaatcttatacttccaacgaataagagggagtatatcaaaacagagtaacaataaacttttgctatgacaccttttctttctttcaaagataaaagaataaggcttttctatagtagtcgagcaaatgttggaataaggaggtatggaattttgaaaatagcctgagaaattcagatcaatgatatataactgttgtcttcaaaaggtcttcaagggaagaaaatttccgatcggaagtccagaataaataccacaagtatagcacaataaacaacagcacaacaacaataataacaacacctgtagcgaaaacgttttcctatttttaaggcgttgttctttgaaaacctgtggcgaagtaaaacatgaaaacaaatgaaaacaccgccaaaccaagaaaagaacaacgaaaaaatatcacttttatttagttcacaacggctaactatcgacgttcacccttcctcagtctatcacatcgtccttagctcgaacaacgccgataggcatcaagttacattgagctttactgcacgttcccgcatgatgccattgactagggcccgccctttcggcaatcattctagcatgttccgcatgttc

SEQ ID NO: 4 - DNA, 222 bp, Artificial Sequence
  Artificial terminator
gtgcaccttttttttctccttccagtgcattatgcaatagacagcacgagtctttgaaaaagtaacttataaaactgtatcaatttttaaacctaaatagattcataaactattcgttaatataaagtgttctaaactatgatgaaaaaataagcagaaaagactaataattcttagttaaaagcactttacaacttgtcaccgtggtggaagttttcaccg

SEQ ID NO: 5 - protein, 894 aa, Saccharomyces cerevisiae [sequence omitted]